European Patent Application EP 4 357 450 A1, published April 24, 2024. Title: Production of recombinant human α-thrombin in plant-based system and the application thereof. Applicant: PROVIEW-MBD Biotech Co., Ltd. Application IB US 63/417261, filed October 18, 2022. The sequence listing filed with the application follows.

SEQUENCE LISTING (1 sequence)

SEQ ID NO: 1 - protein, 313 aa, Homo sapiens
MHHHHHHHHNPIRLIDGRTFGSGEADCGLRPLFEKKSLEDKTERELLESYIDGRIVEGSDAEIGMSPWQVMLFRKSPQELLCGASLISDRWVLTAAHCLLYPPWDKNFTENDLLVRIGKHSRTRYERNIEKISMLEKIYIHPRYNWRENLDRDIALMKLKKPVAFSDYIHPVCLPDRETAASLLQAGYKGRVTGWGNLKETWTANVGKGQPSVLQVVNLPIVERPVCKDSTRIRITDNMFCAGYKPDEGKRGDACEGDSGGPFVMKSPFNNRWYQMGIVSWGEGCDRDGKYGFYTHVFRLKKWIQKVIDQFGE